European Patent Specification EP 4 060 044 B1, published March 13, 2024. Title: Novel cyanate transporter family protein variant and a method for producing L-tryptophan using the same. Applicant: CJ CheilJedang Corporation. The sequence listing filed with the application follows.

SEQUENCE LISTING (10 sequences)

SEQ ID NO: 1 - protein, 384 aa, Artificial Sequence
  cynX
MLLVLVLIGLNMRPLLTSVGPLLPQLRQASGMSFSVAALLTALPVVTMGGLALAGSWLHQHVSERRSVAISLLLIAVGALMRELYPQSALLLSSALLGGVGIGIIQAVMPSVIKRRFQQRTPLVMGLWSAALMGGGGLGAAITPWLVQHSETWYQTLAWWALPAVVALFAWWWQSAREVASSHKTTTTPVRVVFTPRAWTLGVYFGLINGGYASLIAWLPAFYIEIGASAQYSGSLLALMTLGQAAGALLMPAMARHQNRRKLLMLALVLQLVGFCGFIWLPMQLPVLWAMVCGLGLGGAFPLCLLLALDHSVQPAIAGKLVAFMQGIGFIIAGLAPWFSGVLRSISGNYLMDWAFHALCVVGLMIITLRFAPVRFPQLWVKEA

SEQ ID NO: 2 - DNA, 1155 bp, Artificial Sequence
  cynX
atgctgctggtactggtgctgattggtcttaatatgcgaccactgctcacctccgtcgggccactgctaccgcaattgcgccaggcgagcggaatgagctttagcgtggctgccctgttgaccgctctgccggtggttaccatgggcgggctggcgctggccggaagctggcttcatcagcatgtcagcgaacgtcgcagtgtcgccatcagtctgttgctgattgccgtcggtgcattgatgcgtgagctttacccgcaaagtgcgctgctgcttagcagcgcactgcttggtggggtggggatcggcatcattcaggcggtgatgccttcggtgattaaacggcggtttcagcagcgcacgccactggtgatggggctgtggtccgcggctctgatgggcggcggtgggcttggtgccgccataacgccctggttagttcaacatagcgaaacctggtatcaaacactcgcctggtgggcgctgcctgccgttgttgcgctctttgcctggtggtggcaaagcgcccgcgaggtcgcctcttcccacaagacaacaaccactccggttcgcgtggtattcactccccgcgcgtggacgctgggtgtttacttcggtctgattaacggcggttacgccagcctgattgcctggttacccgctttctatattgagattggtgccagcgcgcagtacagcggttccttactggcattgatgacgcttgggcaagccgcaggagctttgctgatgcctgctatggctcgccatcagaatcggcgcaaactgttaatgctggcgctggtgttacaactggtggggttctgcggctttatctggctgccgatgcaattgccggtattgtgggcgatggtgtgtgggttaggtctgggcggcgcgtttccgctctgtttgctgctggcgctcgatcactctgtgcaaccggctattgctggcaagctggtggcgtttatgcagggaatcggttttatcatcgccgggcttgccccgtggttttctggcgtgctgcgtagtatcagcggcaattacctgatggactgggcatttcatgcgctgtgcgtcgttgggctgatgatcataaccctgcgttttgcaccagtacgttttccgcagctgtgggtcaaagaggcatga

SEQ ID NO: 3 - protein, 384 aa, Unknown
  cynX
MLLVLVLIGLNMRPLLTSVGPLLPQLRQASGMSFSVAALLTALPVVTMGGLALAGSWLHQHVSERRSVAISLLLIAVGALMRELYPQSALLLSSALLGGVGIGIIQAVMPSVIKRRFQQRTPLVMGLWSAALMGGGGLGAAITPWLVQHSETWYQTLAWWALPAVVALFAWWWQSAREVASSHKTTTTPVRVVFTPRAWTLGVYFGLINGGYASLIAWLPAFYIEIGASAQYSGSLLALMTLGQAAGALLMPAMARHQDRRKLLMLALVLQLVGFCGFIWLPMQLPVLWAMVCGLGLGGAFPLCLLLALDHSVQPAIAGKLVAFMQGIGFIIAGLAPWFSGVLRSISGNYLMDWAFHALCVVGLMIITLRFAPVRFPQLWVKEA

SEQ ID NO: 4 - DNA, 1155 bp, Unknown
  cynX
atgctgctggtactggtgctgattggtcttaatatgcgaccactgctcacctccgtcgggccactgctaccgcaattgcgccaggcgagcggaatgagctttagcgtggctgccctgttgaccgctctgccggtggttaccatgggcgggctggcgctggccggaagctggcttcatcagcatgtcagcgaacgtcgcagtgtcgccatcagtctgttgctgattgccgtcggtgcattgatgcgtgagctttacccgcaaagtgcgctgctgcttagcagcgcactgcttggtggggtggggatcggcatcattcaggcggtgatgccttcggtgattaaacggcggtttcagcagcgcacgccactggtgatggggctgtggtccgcggctctgatgggcggcggtgggcttggtgccgccataacgccctggttagttcaacatagcgaaacctggtatcaaacactcgcctggtgggcgctgcctgccgttgttgcgctctttgcctggtggtggcaaagcgcccgcgaggtcgcctcttcccacaagacaacaaccactccggttcgcgtggtattcactccccgcgcgtggacgctgggtgtttacttcggtctgattaacggcggttacgccagcctgattgcctggttacccgctttctatattgagattggtgccagcgcgcagtacagcggttccttactggcattgatgacgcttgggcaagccgcaggagctttgctgatgcctgctatggctcgccatcaggatcggcgcaaactgttaatgctggcgctggtgttacaactggtggggttctgcggctttatctggctgccgatgcaattgccggtattgtgggcgatggtgtgtgggttaggtctgggcggcgcgtttccgctctgtttgctgctggcgctcgatcactctgtgcaaccggctattgctggcaagctggtggcgtttatgcagggaatcggttttatcatcgccgggcttgccccgtggttttctggcgtgctgcgtagtatcagcggcaattacctgatggactgggcatttcatgcgctgtgcgtcgttgggctgatgatcataaccctgcgttttgcaccagtacgttttccgcagctgtgggtcaaagaggcatga

SEQ ID NO: 5 - DNA, 40 bp, Artificial Sequence
  Forward Primer
ggaattcgagctcggtacccatgctgctggtactggtgct

SEQ ID NO: 6 - DNA, 21 bp, Artificial Sequence
  Reverse Primer
ttgcgccgattctgatggcga

SEQ ID NO: 7 - DNA, 21 bp, Artificial Sequence
  Forward Primer
tcgccatcagaatcggcgcaa

SEQ ID NO: 8 - DNA, 40 bp, Artificial Sequence
  Reverse Primer
gttatccctagcggatcccctcatgcctctttgacccaca

SEQ ID NO: 9 - DNA, 20 bp, Artificial Sequence
  Forward Primer
atgcgcaaccatcaaaagac

SEQ ID NO: 10 - DNA, 20 bp, Artificial Sequence
  Reverse Primer
gccgcatccggcatgaacaa